European Patent Specification EP 3 881 861 B1, published July 31, 2024. Title: DOSAGE REGIMES FOR THE ADMINISTRATION OF GLUCAGON-LIKE-PEPTIDE-2 (GLP-2) ANALOGUES. Applicant: ZEALAND PHARMA A/S. Application Divisional of EPA 18734135.9. The sequence listing filed with the application follows.

SEQUENCE LISTING (9 sequences)

SEQ ID NO: 1 - protein, 39 aa, Artificial Sequence
  Synthetic peptide sequence
HGEGTFSSELATILDALAARDFIAWLIATKITDKKKKKK

SEQ ID NO: 2 - protein, 36 aa, Artificial Sequence
  Synthetic peptide sequence
HGEGTFSSELATILDALAARDFIAWLIATKITDKKK

SEQ ID NO: 3 - protein, 35 aa, Artificial Sequence
  Synthetic peptide sequence
HGEGTFSSELATILDALAARDFIAWLIATKITDKK

SEQ ID NO: 4 - protein, 34 aa, Artificial Sequence
  Synthetic peptide sequence
HGEGTFSSELATILDALAARDFIAWLIATKITDK

SEQ ID NO: 5 - protein, 33 aa, Artificial Sequence
  Synthetic peptide sequence
HGEGTFSSELATILDALAARDFIAWLIATKITD

SEQ ID NO: 6 - protein, 33 aa, Artificial Sequence; identical to SEQ ID NO: 5
  Synthetic peptide sequence

SEQ ID NO: 7 - protein, 39 aa, Artificial Sequence
  Synthetic peptide sequence
HGEGSFSSELSTILDALAARDFIAWLIATKITDKKKKKK

SEQ ID NO: 8 - protein, 33 aa, Artificial Sequence
  Synthetic peptide sequence
HGEGSFSSELSTILDALAARDFIAWLIATKITD

SEQ ID NO: 9 - protein, 34 aa, Artificial Sequence
  Synthetic peptide sequence
HGEGSFSSELSTILDALAARDFIAWLIATKITDK